European Patent Application EP 4 219 553 A1, published August 2, 2023. Title: Anti-TIGIT antibody and double antibody and their application. Applicant: Nanjing Sanhome Pharmaceutical Co., Ltd. Application EP21871470.7. The sequence listing filed with the application follows.

SEQUENCE LISTING (111 sequences)

SEQ ID NO: 1 - protein, 10 aa, Mus musculus
  HCDR1
GDSITSGYWN

SEQ ID NO: 2 - protein, 16 aa, Mus musculus
  HCDR2
YISYTGSTYYNLSLKS

SEQ ID NO: 3 - protein, 10 aa, Mus musculus
  HCDR3
YILWLRHFDY

SEQ ID NO: 4 - protein, 10 aa, Mus musculus
  HCDR1
GYSITSDYWN

SEQ ID NO: 5 - protein, 16 aa, Mus musculus
  HCDR2
YISYTGSTYYNPSLKR

SEQ ID NO: 6 - protein, 10 aa, Mus musculus
  HCDR3
YRDWPGYFDV

SEQ ID NO: 7 - protein, 10 aa, Mus musculus
  HCDR1
GYTFTRNTMH

SEQ ID NO: 8 - protein, 17 aa, Mus musculus
  HCDR2
FIDPHNTYTRYNQKFKD

SEQ ID NO: 9 - protein, 5 aa, Mus musculus
  HCDR3
WPMDY

SEQ ID NO: 10 - protein, 10 aa, Mus musculus
  HCDR1
GYSFTSNWMN

SEQ ID NO: 11 - protein, 17 aa, Mus musculus
  HCDR2
MIHLYDSETKLNPNFQD

SEQ ID NO: 12 - protein, 9 aa, Mus musculus
  HCDR3
SAGNYRFAY

SEQ ID NO: 13 - protein, 17 aa, Mus musculus
  LCDR1
KSSQSLLYSSNQKNSLA

SEQ ID NO: 14 - protein, 7 aa, Mus musculus
  LCDR2
WASTRES

SEQ ID NO: 15 - protein, 9 aa, Mus musculus
  LCDR3
QQYYGYPLT

SEQ ID NO: 16 - protein, 11 aa, Mus musculus
  LCDR1
RASKSIRKFLA

SEQ ID NO: 17 - protein, 7 aa, Mus musculus
  LCDR2
SGSTLQS

SEQ ID NO: 18 - protein, 9 aa, Mus musculus
  LCDR3
QHYNEYPFT

SEQ ID NO: 19 - protein, 17 aa, Mus musculus
  LCDR1
KSSQSLSWSENQNNYLS

SEQ ID NO: 20 - protein, 7 aa, Mus musculus
  LCDR2
GASIRES

SEQ ID NO: 21 - protein, 11 aa, Mus musculus
  LCDR3
QHNHGSFLPYT

SEQ ID NO: 22 - protein, 11 aa, Mus musculus
  LCDR1
KASQSVSNEVA

SEQ ID NO: 23 - protein, 7 aa, Mus musculus
  LCDR2
SASSRYT

SEQ ID NO: 24 - protein, 9 aa, Mus musculus
  LCDR3
QQHYSSPLT

SEQ ID NO: 25 - protein, 7 aa, Mus musculus
  HCDR1
TYGLGVG

SEQ ID NO: 26 - protein, 16 aa, Mus musculus
  HCDR2
NIWWDDDEYYNPSLKN

SEQ ID NO: 27 - protein, 16 aa, Mus musculus
  HCDR3
IARPHYYWDGRYILDV

SEQ ID NO: 28 - protein, 5 aa, Mus musculus
  HCDR1
DHWMS

SEQ ID NO: 29 - protein, 17 aa, Mus musculus
  HCDR2
NIQYDGSYTNYAPSLKN

SEQ ID NO: 30 - protein, 17 aa, Mus musculus
  HCDR3
GHFRITMASMGASASVY

SEQ ID NO: 31 - protein, 16 aa, Mus musculus
  LCDR1
RSSKSLLHSNGITYLS

SEQ ID NO: 32 - protein, 7 aa, Mus musculus
  LCDR2
QISNLAS

SEQ ID NO: 33 - protein, 9 aa, Mus musculus
  LCDR3
MQFLEVPYT

SEQ ID NO: 34 - protein, 11 aa, Mus musculus
  LCDR1
RTSQDIGNSLR

SEQ ID NO: 35 - protein, 7 aa, Mus musculus
  LCDR2
GATNLAN

SEQ ID NO: 36 - protein, 9 aa, Mus musculus
  LCDR3
LQHNEYPLT

SEQ ID NO: 37 - protein, 118 aa, Mus musculus
  Heavy chain variable region
EVQLQESGPSLVKPSQTLSLTCSVTGDSITSGYWNWIRKFPGNKLEYMGYISYTGSTYYNLSLKSRISITRDTSKNQYYLQLNSVTTEDTATYYCARYILWLRHFDYWGQGTTLTVSS

SEQ ID NO: 38 - protein, 118 aa, Mus musculus
  Heavy chain variable region
EVQLQESGPGLAKPSQTLSLTCSVTGYSITSDYWNWIRKFPGNKLEYMGYISYTGSTYYNPSLKRRVSITRDTSKNNYYLQLNSVTTEDTATYYCARYRDWPGYFDVWGAGTTVTVSS

SEQ ID NO: 39 - protein, 114 aa, Mus musculus
  Heavy chain variable region
QVQLQQSGAELARPGASVKMSCKASGYTFTRNTMHWIKQRPGQGLEWIGFIDPHNTYTRYNQKFKDRATLTADKSSSTAYMQLSSLSSEDSAVYYCARWPMDYWGQGTSVTVSS

SEQ ID NO: 40 - protein, 118 aa, Mus musculus
  Heavy chain variable region
QVQLQQPGAELVRPGTSVNLSCKASGYSFTSNWMNWVKQRPGQGLEWIGMIHLYDSETKLNPNFQDKATLTVDKSSSIAYMQLSSPTSEDSAVYYCARSAGNYRFAYWGQGTLVTVSA

SEQ ID NO: 41 - protein, 113 aa, Mus musculus
  Light chain variable region
DIVMSQSPSSLAVSVGEKVTMSCKSSQSLLYSSNQKNSLAWYQQKPGQSPKLLIYWASTRESGVPDRFTGSGSGTDFTLTISSVKAEDLAVYYCQQYYGYPLTFGAGTKLELK

SEQ ID NO: 42 - protein, 107 aa, Mus musculus
  Light chain variable region
DVQITQSPSYLAASPGETITINCRASKSIRKFLAWYQEKPGKTNKLLIYSGSTLQSGIPSRFSGSGSGTDFTLTISTLEPEDFAVYYCQHYNEYPFTFGGGTKLEIK

SEQ ID NO: 43 - protein, 115 aa, Mus musculus
  Light chain variable region
DIVMTQFPSSLAVTAGEKVTMRCKSSQSLSWSENQNNYLSWYQQKQGQPPKLLIYGASIRESWVPDRFTGSGSGTDFTLTISNVHAEDLGVYFCQHNHGSFLPYTFGGGTKLEIK

SEQ ID NO: 44 - protein, 107 aa, Mus musculus
  Light chain variable region
SIVMTQTPKFLPVTAEDRVTITCKASQSVSNEVAWYQQKPGQSPKLLIYSASSRYTGVPDRFIGGGSATDFTFTISSVQVEDLAVYFCQQHYSSPLTFGAGTKLELK

SEQ ID NO: 45 - protein, 99 aa, Artificial Sequence
  Heavy chain variable region
QVQLQESGPGLVKPSQTLSLTCTVSGGSISSGGYYWSWIRQHPGKGLEWIGYIYYSGSTYYNPSLKSRVTISVDTSKNQFSLKLSSVTAADTAVYYCAR

SEQ ID NO: 46 - protein, 98 aa, Artificial Sequence
  Heavy chain variable region
QVQLVQSGAEVKKPGASVKVSCKASGYTFTSYAMHWVRQAPGQRLEWMGWINAGNGNTKYSQKFQGRVTITRDTSASTAYMELSSLRSEDTAVYYCAR

SEQ ID NO: 47 - protein, 101 aa, Artificial Sequence
  Light chain variable region
DIVMTQSPDSLAVSLGERATINCKSSQSVLYSSNNKNYLAWYQQKPGQPPKLLIYWASTRESGVPDRFSGSGSGTDFTLTISSLQAEDVAVYYCQQYYSTP

SEQ ID NO: 48 - protein, 118 aa, Artificial Sequence
  Heavy chain variable region
QVQLQESGPGLVKPSQTLSLTCTVSGDSITSGYWNWIRQHPGKGLEWIGYISYTGSTYYNLSLKSRVTISVDTSKNQFSLKLSSVTAADTAVYYCARYILWLRHFDYWGQGTLVTVSS

SEQ ID NO: 49 - protein, 118 aa, Artificial Sequence
  Heavy chain variable region
QVQLQESGPGLVKPSQTLSLTCTVSGDSITSGYWNWIRQHPGKGLEYIGYISYTGSTYYNLSLKSRVTISVDTSKNQFSLKLSSVTAADTAVYYCARYILWLRHFDYWGQGTLVTVSS

SEQ ID NO: 50 - protein, 118 aa, Artificial Sequence
  Heavy chain variable region
QVQLQESGPGLVKPSQTLSLTCTVSGDSITSGYWNWIRQHPGKGLEYIGYISYTGSTYYNLSLKSRVTISRDTSKNQFSLKLSSVTAADTAVYYCARYILWLRHFDYWGQGTLVTVSS

SEQ ID NO: 51 - protein, 118 aa, Artificial Sequence
  Heavy chain variable region
QVQLQESGPGLVKPSQTLSLTCTVSGDSITSGYWNWIRQHPGKGLEYIGYISYTGSTYYNLSLKSRITISRDTSKNQYSLKLSSVTAADTAVYYCARYILWLRHFDYWGQGTLVTVSS

SEQ ID NO: 52 - protein, 118 aa, Artificial Sequence
  Heavy chain variable region
QVQLQESGPGLVKPSQTLSLTCTVSGDSITSGYWNWIRQHPGKGLEYMGYISYTGSTYYNLSLKSRITISRDTSKNQYSLKLSSVTAADTAVYYCARYILWLRHFDYWGQGTLLTVSS

SEQ ID NO: 53 - protein, 113 aa, Artificial Sequence
  Light chain variable region
DIVMTQSPDSLAVSLGERATINCKSSQSLLYSSNQKNSLAWYQQKPGQPPKLLIYWASTRESGVPDRFSGSGSGTDFTLTISSLQAEDVAVYYCQQYYGYPLTFGGGTKLEIK

SEQ ID NO: 54 - protein, 113 aa, Artificial Sequence
  Light chain variable region
DIVMTQSPDSLAVSLGERATISCKSSQSLLYSSNQKNSLAWYQQKPGQPPKLLIYWASTRESGVPDRFSGSGSGTDFTLTISSLQAEDVAVYYCQQYYGYPLTFGGGTKLEIK

SEQ ID NO: 55 - protein, 113 aa, Artificial Sequence
  Light chain variable region
DIVMTQSPDSLAVSLGERVTISCKSSQSLLYSSNQKNSLAWYQQKPGQPPKLLIYWASTRESGVPDRFSGSGSGTDFTLTISSVQAEDVAVYYCQQYYGYPLTFGGGTKLEIK

SEQ ID NO: 56 - protein, 113 aa, Artificial Sequence
  Light chain variable region
DIVMTQSPDSLAVSLGERVTMSCKSSQSLLYSSNQKNSLAWYQQKPGQPPKLLIYWASTRESGVPDRFSGSGSGTDFTLTISSVQAEDVAVYYCQQYYGYPLTFGGGTKLEIK

SEQ ID NO: 57 - protein, 114 aa, Artificial Sequence
  Heavy chain variable region
QVQLVQSGAEVKKPGASVKVSCKASGYTFTRNTMHWVRQAPGQRLEWMGFIDPHNTYTRYNQKFKDRVTITRDTSASTAYMELSSLRSEDTAVYYCARWPMDYWGQGTLVTVSS

SEQ ID NO: 58 - protein, 114 aa, Artificial Sequence
  Heavy chain variable region
QVQLVQSGAEVKKPGASVKVSCKASGYTFTRNTMHWVRQAPGQRLEWMGFIDPHNTYTRYNQKFKDRVTITADTSASTAYMELSSLRSEDTAVYYCARWPMDYWGQGTLVTVSS

SEQ ID NO: 59 - protein, 114 aa, Artificial Sequence
  Heavy chain variable region
QVQLVQSGAEVKKPGASVKVSCKASGYTFTRNTMHWIRQAPGQRLEWMGFIDPHNTYTRYNQKFKDRVTITADTSASTAYMELSSLRSEDTAVYYCARWPMDYWGQGTLVTVSS

SEQ ID NO: 60 - protein, 114 aa, Artificial Sequence
  Heavy chain variable region
QVQLVQSGAEVAKPGASVKVSCKASGYTFTRNTMHWIRQAPGQRLEWIGFIDPHNTYTRYNQKFKDRATITADTSASTAYMELSSLRSEDTAVYYCARWPMDYWGQGTLVTVSS

SEQ ID NO: 61 - protein, 114 aa, Artificial Sequence
  Heavy chain variable region
QVQLVQSGAEVAKPGASVKMSCKASGYTFTRNTMHWIKQAPGQRLEWIGFIDPHNTYTRYNQKFKDRATLTADTSASTAYMELSSLRSEDTAVYYCARWPMDYWGQGTLVTVSS

SEQ ID NO: 62 - protein, 115 aa, Artificial Sequence
  Light chain variable region
DIVMTQSPDSLAVSLGERATINCKSSQSLSWSENQNNYLSWYQQKPGQPPKLLIYGASIRESGVPDRFSGSGSGTDFTLTISSLQAEDVAVYYCQHNHGSFLPYTFGQGTKLEIK

SEQ ID NO: 63 - protein, 115 aa, Artificial Sequence
  Light chain variable region
DIVMTQSPDSLAVSLGERVTINCKSSQSLSWSENQNNYLSWYQQKPGQPPKLLIYGASIRESGVPDRFSGSGSGTDFTLTISSVQAEDVGVYYCQHNHGSFLPYTFGQGTKLEIK

SEQ ID NO: 64 - protein, 115 aa, Artificial Sequence
  Light chain variable region
DIVMTQSPDSLAVSLGERVTMRCKSSQSLSWSENQNNYLSWYQQKPGQPPKLLIYGASIRESGVPDRFSGSGSGTDFTLTISSVQAEDVGVYYCQHNHGSFLPYTFGQGTKLEIK

SEQ ID NO: 65 - protein, 378 aa, Artificial Sequence
  TIGIT-hIgG1-Fc fusion protein
MRWCLLLIWAQGLRQAPLASGMMTGTIETTGNISAEKGGSIILQCHLSSTTAQVTQVNWEQQDQLLAICNADLGWHISPSFKDRVAPGPGLGLTLQSLTVNDTGEYFCIYHTYPDGTYTGRIFLEVLESSVAEHGARFQIPIEGRMDPKSCDKTHTCPPCPAPELLGGPSVFLFPPKPKDTLMISRTPEVTCVVVDVSHEDPEVKFNWYVDGVEVHNAKTKPREEQYNSTYRVVSVLTVLHQDWLNGKEYKCKVSNKALPAPIEKTISKAKGQPREPQVYTLPPSRDELTKNQVSLTCLVKGFYPSDIAVEWESNGQPENNYKTTPPVLDSDGSFFLYSKLTVDKSRWQQGNVFSCSVMHEALHNHYTQKSLSLSPGK

SEQ ID NO: 66 - protein, 377 aa, Artificial Sequence
  TIGIT-mIgG1-Fc fusion protein
MRWCLLLIWAQGLRQAPLASGMMTGTIETTGNISAEKGGSIILQCHLSSTTAQVTQVNWEQQDQLLAICNADLGWHISPSFKDRVAPGPGLGLTLQSLTVNDTGEYFCIYHTYPDGTYTGRIFLEVLESSVAEHGARFQIPFSPEPRGPTIKPCPPCKCPAPNLLGGPSVFIFPPKIKDVLMISLSPIVTCVVVDVSEDDPDVQISWFVNNVEVHTAQTQTHREDYNSTLRVVSALPIQHQDWMSGKEFKCKVNNKDLPAPIERTISKPKGSVRAPQVYVLPPPEEEMTKKQVTLTCMVTDFMPEDIYVEWTNNGKTELNYKNTEPVLDSDGSYFMYSKLRVEKKNWVERNSYSCSVVHEGLHNHHTTKSFSRTPGK

SEQ ID NO: 67 - protein, 150 aa, Artificial Sequence
  TIGIT-his fusion protein
MRWCLLLIWAQGLRQAPLASGMMTGTIETTGNISAEKGGSIILQCHLSSTTAQVTQVNWEQQDQLLAICNADLGWHISPSFKDRVAPGPGLGLTLQSLTVNDTGEYFCIYHTYPDGTYTGRIFLEVLESSVAEHGARFQIPSGSHHHHHH

SEQ ID NO: 68 - protein, 580 aa, Artificial Sequence
  CD155-hIgG1-Fc fusion protein
MARAMAAAWPLLLVALLVLSWPPPGTGDVVVQAPTQVPGFLGDSVTLPCYLQVPNMEVTHVSQLTWARHGESGSMAVFHQTQGPSYSESKRLEFVAARLGAELRNASLRMFGLRVEDEGNYTCLFVTFPQGSRSVDIWLRVLAKPQNTAEVQKVQLTGEPVPMARCVSTGGRPPAQITWHSDLGGMPNTSQVPGFLSGTVTVTSLWILVPSSQVDGKNVTCKVEHESFEKPQLLTVNLTVYYPPEVSISGYDNNWYLGQNEATLTCDARSNPEPTGYNWSTTMGPLPPFAVAQGAQLLIRPVDKPINTTLICNVTNALGARQAELTVQVKEGPPSEHSGMSRNIEGRMDPKSCDKTHTCPPCPAPELLGGPSVFLFPPKPKDTLMISRTPEVTCVVVDVSHEDPEVKFNWYVDGVEVHNAKTKPREEQYNSTYRVVSVLTVLHQDWLNGKEYKCKVSNKALPAPIEKTISKAKGQPREPQVYTLPPSRDELTKNQVSLTCLVKGFYPSDIAVEWESNGQPENNYKTTPPVLDSDGSFFLYSKLTVDKSRWQQGNVFSCSVMHEALHNHYTQKSLSLSPGK

SEQ ID NO: 69 - protein, 579 aa, Artificial Sequence
  CD155-mIgG1-Fc fusion protein
MARAMAAAWPLLLVALLVLSWPPPGTGDVVVQAPTQVPGFLGDSVTLPCYLQVPNMEVTHVSQLTWARHGESGSMAVFHQTQGPSYSESKRLEFVAARLGAELRNASLRMFGLRVEDEGNYTCLFVTFPQGSRSVDIWLRVLAKPQNTAEVQKVQLTGEPVPMARCVSTGGRPPAQITWHSDLGGMPNTSQVPGFLSGTVTVTSLWILVPSSQVDGKNVTCKVEHESFEKPQLLTVNLTVYYPPEVSISGYDNNWYLGQNEATLTCDARSNPEPTGYNWSTTMGPLPPFAVAQGAQLLIRPVDKPINTTLICNVTNALGARQAELTVQVKEGPPSEHSGMSRNFSPEPRGPTIKPCPPCKCPAPNLLGGPSVFIFPPKIKDVLMISLSPIVTCVVVDVSEDDPDVQISWFVNNVEVHTAQTQTHREDYNSTLRVVSALPIQHQDWMSGKEFKCKVNNKDLPAPIERTISKPKGSVRAPQVYVLPPPEEEMTKKQVTLTCMVTDFMPEDIYVEWTNNGKTELNYKNTEPVLDSDGSYFMYSKLRVEKKNWVERNSYSCSVVHEGLHNHHTTKSFSRTPGK

SEQ ID NO: 70 - protein, 349 aa, Artificial Sequence
  CD155-his fusion protein
MARAMAAAWPLLLVALLVLSWPPPGTGDVVVQAPTQVPGFLGDSVTLPCYLQVPNMEVTHVSQLTWARHGESGSMAVFHQTQGPSYSESKRLEFVAARLGAELRNASLRMFGLRVEDEGNYTCLFVTFPQGSRSVDIWLRVLAKPQNTAEVQKVQLTGEPVPMARCVSTGGRPPAQITWHSDLGGMPNTSQVPGFLSGTVTVTSLWILVPSSQVDGKNVTCKVEHESFEKPQLLTVNLTVYYPPEVSISGYDNNWYLGQNEATLTCDARSNPEPTGYNWSTTMGPLPPFAVAQGAQLLIRPVDKPINTTLICNVTNALGARQAELTVQVKEGPPSEHSGMSRNHHHHHH

SEQ ID NO: 71 - protein, 130 aa, Artificial Sequence
  Heavy chain variable region of 22G2
QVQLQESGPGLVKPSETLSLTCTVSGGSVSSGIYYWSWIRQPPGKGLEWIGYIYYSGSTNYNPSLKSRVTISVDTSKNQFSLKLSSVTAADTAVYYCARDYYVSGNYYNVDYYFFGVDVWGQGTTVTVSS

SEQ ID NO: 72 - protein, 109 aa, Artificial Sequence
  Light chain variable region of 22G2
EIVLTQSPATLSLSPGERATLSCRASQSVSSYLAWYQQKPGQAPRLLIYDASNRATGIPARFSGSGSGTDFTLTISSLEPEDFAVYYCQQRSNWPPLFTFGPGTKVDIK

SEQ ID NO: 73 - protein, 244 aa, Artificial Sequence
  TIGIT protein
MRWCLLLIWAQGLRQAPLASGMMTGTIETTGNISAEKGGSIILQCHLSSTTAQVTQVNWEQQDQLLAICNADLGWHISPSFKDRVAPGPGLGLTLQSLTVNDTGEYFCIYHTYPDGTYTGRIFLEVLESSVAEHGARFQIPLLGAMAATLVVICTAVIVVVALTRKKKALRIHSVEGDLRRKSAGQEEWSPSAPSPPGSCVQAEAAPAGLCGEQRGEDCAELHDYFNVLSYRSLGNCSFFTETG

SEQ ID NO: 74 - protein, 417 aa, Artificial Sequence
  CD155 protein
MARAMAAAWPLLLVALLVLSWPPPGTGDVVVQAPTQVPGFLGDSVTLPCYLQVPNMEVTHVSQLTWARHGESGSMAVFHQTQGPSYSESKRLEFVAARLGAELRNASLRMFGLRVEDEGNYTCLFVTFPQGSRSVDIWLRVLAKPQNTAEVQKVQLTGEPVPMARCVSTGGRPPAQITWHSDLGGMPNTSQVPGFLSGTVTVTSLWILVPSSQVDGKNVTCKVEHESFEKPQLLTVNLTVYYPPEVSISGYDNNWYLGQNEATLTCDARSNPEPTGYNWSTTMGPLPPFAVAQGAQLLIRPVDKPINTTLICNVTNALGARQAELTVQVKEGPPSEHSGMSRNAIIFLVLGILVFLILLGIGIYFYWSKCSREVLWHCHLCPSSTEHASASANGHVSYSAVSRENSSSQDPQTEGTR

SEQ ID NO: 75 - protein, 126 aa, Artificial Sequence
  Heavy chain variable region
QVTLKESGPGILQPSQTLSLTCTFSGFSLRTYGLGVGWIRQLSGKGLEWLANIWWDDDEYYNPSLKNRLTISKDTSNNQAFLKITNVDTADTATYYCARIARPHYYWDGRYILDVWGQGASVTVSS

SEQ ID NO: 76 - protein, 126 aa, Artificial Sequence
  Heavy chain variable region
EVQLVESEGGLVQPGASVKLSCVGSGFSFSDHWMSWVRQTPGKTMEWIGNIQYDGSYTNYAPSLKNRFTISRDNAKNTLYLQMTNLRSEDTATYYCTRGHFRITMASMGASASVYWGQGVMVTVSS

SEQ ID NO: 77 - protein, 112 aa, Artificial Sequence
  Light chain variable region
DIMMTQSPLSVAVTPGESASISCRSSKSLLHSNGITYLSWYLQRPEKSPQLLIFQISNLASGVSDRFSGSGSGTDFTLIISKVETEDVGIYYCMQFLEVPYTFGAGTKLELK

SEQ ID NO: 78 - protein, 107 aa, Artificial Sequence
  Light chain variable region
DIQMTQSPSSLPTSLGDRVTITCRTSQDIGNSLRWFQQKPGKSPRLMIHGATNLANGVPSRFSGSRAGSDYSLTINSLESEDMAMYYCLQHNEYPLTFGSGTKLEIK

SEQ ID NO: 79 - protein, 126 aa, Artificial Sequence
  Heavy chain variable region
QVTLKESGPVLVKPTETLTLTCTVSGFSLSTYGLGVGWIRQPPGKALEWLANIWWDDDEYYNPSLKNRLTISKDTSKSQVVLTMTNMDPVDTATYYCARIARPHYYWDGRYILDVWGQGTTVTVSS

SEQ ID NO: 80 - protein, 126 aa, Artificial Sequence
  Heavy chain variable region
QVTLKESGPVLVKPTETLTLTCTFSGFSLSTYGLGVGWIRQPPGKALEWLANIWWDDDEYYNPSLKNRLTISKDTSKSQAVLTMTNMDPVDTATYYCARIARPHYYWDGRYILDVWGQGTTVTVSS

SEQ ID NO: 81 - protein, 126 aa, Artificial Sequence
  Heavy chain variable region
QVTLKESGPVLVKPTETLTLTCTFSGFSLRTYGLGVGWIRQPPGKALEWLANIWWDDDEYYNPSLKNRLTISKDTSKSQAVLTMTNMDPVDTATYYCARIARPHYYWDGRYILDVWGQGTTVTVSS

SEQ ID NO: 82 - protein, 126 aa, Artificial Sequence
  Heavy chain variable region
QVTLKESGPVLVKPTETLTLTCTFSGFSLSTYGLGVGWIRQPPGKALEWLANIWWDDDEYYNPSLKNRLTISKDTSKSQAVLTITNVDPVDTATYYCARIARPHYYWDGRYILDVWGQGTTVTVSS

SEQ ID NO: 83 - protein, 126 aa, Artificial Sequence
  Heavy chain variable region
QVTLKESGPVLVKPTETLTLTCTFSGFSLRTYGLGVGWIRQPPGKALEWLANIWWDDDEYYNPSLKNRLTISKDTSKSQAVLTITNVDPVDTATYYCARIARPHYYWDGRYILDVWGQGTTVTVSS

SEQ ID NO: 84 - protein, 112 aa, Artificial Sequence
  Light chain variable region
DIVMTQSPLSLPVTPGEPASISCRSSKSLLHSNGITYLSWYLQKPGQSPQLLIYQISNLASGVPDRFSGSGSGTDFTLKISRVEAEDVGVYYCMQFLEVPYTFGQGTKLEIK

SEQ ID NO: 85 - protein, 112 aa, Artificial Sequence
  Light chain variable region
DIVMTQSPLSLPVTPGEPASISCRSSKSLLHSNGITYLSWYLQKPGQSPQLLIFQISNLASGVPDRFSGSGSGTDFTLKISRVEAEDVGVYYCMQFLEVPYTFGQGTKLEIK

SEQ ID NO: 86 - protein, 112 aa, Artificial Sequence
  Light chain variable region
DIVMTQSPLSLPVTPGEPASISCRSSKSLLHSNGITYLSWYLQKPEKSPQLLIFQISNLASGVPDRFSGSGSGTDFTLKISRVEAEDVGVYYCMQFLEVPYTFGQGTKLEIK

SEQ ID NO: 87 - protein, 112 aa, Artificial Sequence
  Light chain variable region
DIVMTQSPLSLPVTPGEPASISCRSSKSLLHSNGITYLSWYLQKPEKSPQLLIFQISNLASGVPDRFSGSGSGTDFTLKISRVEAEDVGIYYCMQFLEVPYTFGQGTKLEIK

SEQ ID NO: 88 - protein, 126 aa, Artificial Sequence
  Heavy chain variable region
EVQLVESGGGLVQPGGSLRLSCAASGFTFSDHWMSWVRQAPGKGLEWVANIQYDGSYTNYAPSLKNRFTISRDNAKNSLYLQMNSLRAEDTAVYYCARGHFRITMASMGASASVYWGQGTMVTVSS

SEQ ID NO: 89 - protein, 126 aa, Artificial Sequence
  Heavy chain variable region
EVQLVESGGGLVQPGGSLRLSCAASGFTFSDHWMSWVRQAPGKGLEWIANIQYDGSYTNYAPSLKNRFTISRDNAKNSLYLQMNSLRAEDTAVYYCARGHFRITMASMGASASVYWGQGTMVTVSS

SEQ ID NO: 90 - protein, 126 aa, Artificial Sequence
  Heavy chain variable region
EVQLVESGGGLVQPGGSLRLSCAASGFTFSDHWMSWVRQAPGKGMEWIANIQYDGSYTNYAPSLKNRFTISRDNAKNSLYLQMNSLRAEDTAVYYCARGHFRITMASMGASASVYWGQGTMVTVSS

SEQ ID NO: 91 - protein, 126 aa, Artificial Sequence
  Heavy chain variable region
EVQLVESGGGLVQPGGSLRLSCAASGFTFSDHWMSWVRQAPGKGMEWIANIQYDGSYTNYAPSLKNRFTISRDNAKNSLYLQMNSLRAEDTAVYYCTRGHFRITMASMGASASVYWGQGTMVTVSS

SEQ ID NO: 92 - protein, 126 aa, Artificial Sequence
  Heavy chain variable region
EVQLVESGGGLVQPGGSLRLSCAASGFTFSDHWMSWVRQAPGKTMEWIGNIQYDGSYTNYAPSLKNRFTISRDNAKNSLYLQMNSLRAEDTATYYCTRGHFRITMASMGASASVYWGQGTMVTVSS

SEQ ID NO: 93 - protein, 107 aa, Artificial Sequence
  Light chain variable region
DIQMTQSPSSLSASVGDRVTITCRTSQDIGNSLRWYQQKPGKAPKLLIYGATNLANGVPSRFSGSGSGTDFTLTISSLQPEDFATYYCLQHNEYPLTFGQGTKLEIK

SEQ ID NO: 94 - protein, 107 aa, Artificial Sequence
  Light chain variable region
DIQMTQSPSSLSASVGDRVTITCRTSQDIGNSLRWYQQKPGKAPKLLIHGATNLANGVPSRFSGSGSGTDFTLTISSLQPEDFATYYCLQHNEYPLTFGQGTKLEIK

SEQ ID NO: 95 - protein, 107 aa, Artificial Sequence; identical to SEQ ID NO: 94
  Light chain variable region

SEQ ID NO: 96 - protein, 107 aa, Artificial Sequence
  Light chain variable region
DIQMTQSPSSLSASVGDRVTITCRTSQDIGNSLRWFQQKPGKAPRLMIHGATNLANGVPSRFSGSGSGTDFTLTISSLQPEDFATYYCLQHNEYPLTFGQGTKLEIK

SEQ ID NO: 97 - protein, 107 aa, Artificial Sequence
  Light chain variable region
DIQMTQSPSSLSASVGDRVTITCRTSQDIGNSLRWFQQKPGKAPRLMIHGATNLANGVPSRFSGSGSGTDFTLTISSLQPEDFAMYYCLQHNEYPLTFGQGTKLEIK

SEQ ID NO: 98 - protein, 126 aa, Artificial Sequence; identical to SEQ ID NO: 81
  Heavy chain variable region of SHS006-T-Hu17-31

SEQ ID NO: 99 - protein, 126 aa, Artificial Sequence; identical to SEQ ID NO: 92
  Heavy chain variable region of SHS006-T-Hu23-53

SEQ ID NO: 100 - protein, 112 aa, Artificial Sequence; identical to SEQ ID NO: 84
  Light chain variable region of SHS006-T-Hu17-31

SEQ ID NO: 101 - protein, 107 aa, Artificial Sequence
  Light chain variable region of SHS006-T-Hu23-53
DIQMTQSPSSLSASVGDRVTITCRTSQDIGNSLRWFQQKPGKAPKLLIHGATNLANGVPSRFSGSGSGTDFTLTISSLQPEDFATYYCLQHNEYPLTFGQGTKLEIK

SEQ ID NO: 102 - protein, 707 aa, Artificial Sequence
  ScFab-T2353-Knob-PHR protein
DIQMTQSPSSLSASVGDRVTITCRTSQDIGNSLRWFQQKPGKAPKLLIHGATNLANGVPSRFSGSGSGTDFTLTISSLQPEDFATYYCLQHNEYPLTFGCGTKLEIKRTVAAPSVFIFPPSDEQLKSGTASVVCLLNNFYPREAKVQWKVDNALQSGNSQESVTEQDSKDSTYSLSSTLTLSKADYEKHKVYACEVTHQGLSSPVTKSFNRGECGGGGSGGGGSGGGGSGGGGSGGGGSGGGGSGGGGSGGGGSEVQLVESGGGLVQPGGSLRLSCAASGFTFSDHWMSWVRQAPGKCMEWIGNIQYDGSYTNYAPSLKNRFTISRDNAKNSLYLQMNSLRAEDTATYYCTRGHFRITMASMGASASVYWGQGTMVTVSSASTKGPSVFPLAPCSRSTSESTAALGCLVKDYFPEPVTVSWNSGALTSGVHTFPAVLQSSGLYSLSSVVTVPSSSLGTKTYTCNVDHKPSNTKVDKRVESKYGPPCPPCPAPEFLGGPSVFLFPPKPKDTLMISRTPEVTCVVVDVSQEDPEVQFNWYVDGVEVHNAKTKPREEQFNSTYRVVSVLTVLHQDWLNGKEYKCKVSNKGLPSSIEKTISKAKGQPREPQVYTLPPCQEEMTKNQVSLWCLVKGFYPSDIAVEWESNGQPENNYKTTPPVLDSDGSFFLYSRLTVDKSRWQEGNVFSCSVMHEALHNHYTQKSLSLSLGK

SEQ ID NO: 103 - protein, 705 aa, Artificial Sequence
  HuPL721-scfab-hole-PHR protein
DIVMTQSPDSLAVSLGERATISCKSSQSLLYSSNQKNSLAWYQQKPGQPPKLLIYWASTRESGVPDRFSGSGSGTDFTLTISSLQAEDVAVYYCQQYYGYPLTFGCGTKLEIKRTVAAPSVFIFPPSDEQLKSGTASVVCLLNNFYPREAKVQWKVDNALQSGNSQESVTEQDSKDSTYSLSSTLTLSKADYEKHKVYACEVTHQGLSSPVTKSFNRGECGGGGSGGGGSGGGGSGGGGSGGGGSGGGGSGGGGSGGGGSQVQLQESGPGLVKPSQTLSLTCTVSGDSITSGYWNWIRQHPGKCLEYIGYISYTGSTYYNLSLKSRVTISRDTSKNQFSLKLSSVTAADTAVYYCARYILWLRHFDYWGQGTLVTVSSASTKGPSVFPLAPCSRSTSESTAALGCLVKDYFPEPVTVSWNSGALTSGVHTFPAVLQSSGLYSLSSVVTVPSSSLGTKTYTCNVDHKPSNTKVDKRVESKYGPPCPPCPAPEFLGGPSVFLFPPKPKDTLMISRTPEVTCVVVDVSQEDPEVQFNWYVDGVEVHNAKTKPREEQFNSTYRVVSVLTVLHQDWLNGKEYKCKVSNKGLPSSIEKTISKAKGQPREPQVCTLPPSQEEMTKNQVSLSCAVKGFYPSDIAVEWESNGQPENNYKTTPPVLDSDGSFFLVSRLTVDKSRWQEGNVFSCSVMHEALHNHYTQKSLSLSLGK

SEQ ID NO: 104 - protein, 708 aa, Artificial Sequence
  PL721-T2353-scFv-HC-PHR protein
QVQLQESGPGLVKPSQTLSLTCTVSGDSITSGYWNWIRQHPGKGLEYIGYISYTGSTYYNLSLKSRVTISRDTSKNQFSLKLSSVTAADTAVYYCARYILWLRHFDYWGQGTLVTVSSASTKGPSVFPLAPCSRSTSESTAALGCLVKDYFPEPVTVSWNSGALTSGVHTFPAVLQSSGLYSLSSVVTVPSSSLGTKTYTCNVDHKPSNTKVDKRVESKYGPPCPPCPAPEFEGGPSVFLFPPKPKDTLMISRTPEVTCVVVDVSQEDPEVQFNWYVDGVEVHNAKTKPREEQFNSTYRVVSVLTVLHQDWLNGKEYKCKVSNKGLPSSIEKTISKAKGQPREPQVYTLPPSQEEMTKNQVSLTCLVKGFYPSDIAVEWESNGQPENNYKTTPPVLDSDGSFFLYSRLTVDKSRWQEGNVFSCSVMHEALHNHYTQKSLSLSLGKGGGGSGGGGSEVQLVESGGGLVQPGGSLRLSCAASGFTFSDHWMSWVRQAPGKCMEWIGNIQYDGSYTNYAPSLKNRFTISRDNAKNSLYLQMNSLRAEDTATYYCTRGHFRITMASMGASASVYWGQGTMVTVSSGGGGSGGGGSGGGGSGGGGSDIQMTQSPSSLSASVGDRVTITCRTSQDIGNSLRWFQQKPGKAPKLLIHGATNLANGVPSRFSGSGSGTDFTLTISSLQPEDFATYYCLQHNEYPLTFGCGTKLEIK

SEQ ID NO: 105 - protein, 220 aa, Artificial Sequence
  HuPL721-VL1-PHR protein
DIVMTQSPDSLAVSLGERATISCKSSQSLLYSSNQKNSLAWYQQKPGQPPKLLIYWASTRESGVPDRFSGSGSGTDFTLTISSLQAEDVAVYYCQQYYGYPLTFGGGTKLEIKRTVAAPSVFIFPPSDEQLKSGTASVVCLLNNFYPREAKVQWKVDNALQSGNSQESVTEQDSKDSTYSLSSTLTLSKADYEKHKVYACEVTHQGLSSPVTKSFNRGEC

SEQ ID NO: 106 - protein, 705 aa, Artificial Sequence
  HuPL743-scfab-hole-PHR protein
DIVMTQSPDSLAVSLGERVTMSCKSSQSLLYSSNQKNSLAWYQQKPGQPPKLLIYWASTRESGVPDRFSGSGSGTDFTLTISSVQAEDVAVYYCQQYYGYPLTFGCGTKLEIKRTVAAPSVFIFPPSDEQLKSGTASVVCLLNNFYPREAKVQWKVDNALQSGNSQESVTEQDSKDSTYSLSSTLTLSKADYEKHKVYACEVTHQGLSSPVTKSFNRGECGGGGSGGGGSGGGGSGGGGSGGGGSGGGGSGGGGSGGGGSQVQLQESGPGLVKPSQTLSLTCTVSGDSITSGYWNWIRQHPGKCLEYMGYISYTGSTYYNLSLKSRITISRDTSKNQYSLKLSSVTAADTAVYYCARYILWLRHFDYWGQGTLLTVSSASTKGPSVFPLAPCSRSTSESTAALGCLVKDYFPEPVTVSWNSGALTSGVHTFPAVLQSSGLYSLSSVVTVPSSSLGTKTYTCNVDHKPSNTKVDKRVESKYGPPCPPCPAPEFLGGPSVFLFPPKPKDTLMISRTPEVTCVVVDVSQEDPEVQFNWYVDGVEVHNAKTKPREEQFNSTYRVVSVLTVLHQDWLNGKEYKCKVSNKGLPSSIEKTISKAKGQPREPQVCTLPPSQEEMTKNQVSLSCAVKGFYPSDIAVEWESNGQPENNYKTTPPVLDSDGSFFLVSRLTVDKSRWQEGNVFSCSVMHEALHNHYTQKSLSLSLGK

SEQ ID NO: 107 - protein, 708 aa, Artificial Sequence
  PL743-T2353-scFv-HC-PHR protein
QVQLQESGPGLVKPSQTLSLTCTVSGDSITSGYWNWIRQHPGKGLEYMGYISYTGSTYYNLSLKSRITISRDTSKNQYSLKLSSVTAADTAVYYCARYILWLRHFDYWGQGTLLTVSSASTKGPSVFPLAPCSRSTSESTAALGCLVKDYFPEPVTVSWNSGALTSGVHTFPAVLQSSGLYSLSSVVTVPSSSLGTKTYTCNVDHKPSNTKVDKRVESKYGPPCPPCPAPEFEGGPSVFLFPPKPKDTLMISRTPEVTCVVVDVSQEDPEVQFNWYVDGVEVHNAKTKPREEQFNSTYRVVSVLTVLHQDWLNGKEYKCKVSNKGLPSSIEKTISKAKGQPREPQVYTLPPSQEEMTKNQVSLTCLVKGFYPSDIAVEWESNGQPENNYKTTPPVLDSDGSFFLYSRLTVDKSRWQEGNVFSCSVMHEALHNHYTQKSLSLSLGKGGGGSGGGGSEVQLVESGGGLVQPGGSLRLSCAASGFTFSDHWMSWVRQAPGKCMEWIGNIQYDGSYTNYAPSLKNRFTISRDNAKNSLYLQMNSLRAEDTATYYCTRGHFRITMASMGASASVYWGQGTMVTVSSGGGGSGGGGSGGGGSGGGGSDIQMTQSPSSLSASVGDRVTITCRTSQDIGNSLRWFQQKPGKAPKLLIHGATNLANGVPSRFSGSGSGTDFTLTISSLQPEDFATYYCLQHNEYPLTFGCGTKLEIK

SEQ ID NO: 108 - protein, 220 aa, Artificial Sequence
  HuPL743-VL3-PHR protein
DIVMTQSPDSLAVSLGERVTMSCKSSQSLLYSSNQKNSLAWYQQKPGQPPKLLIYWASTRESGVPDRFSGSGSGTDFTLTISSVQAEDVAVYYCQQYYGYPLTFGGGTKLEIKRTVAAPSVFIFPPSDEQLKSGTASVVCLLNNFYPREAKVQWKVDNALQSGNSQESVTEQDSKDSTYSLSSTLTLSKADYEKHKVYACEVTHQGLSSPVTKSFNRGEC

SEQ ID NO: 109 - protein, 703 aa, Artificial Sequence
  HuPL1642-scfab-hole-PHR protein
DIVMTQSPDSLAVSLGERVTMRCKSSQSLSWSENQNNYLSWYQQKPGQPPKLLIYGASIRESGVPDRFSGSGSGTDFTLTISSVQAEDVGVYYCQHNHGSFLPYTFGCGTKLEIKRTVAAPSVFIFPPSDEQLKSGTASVVCLLNNFYPREAKVQWKVDNALQSGNSQESVTEQDSKDSTYSLSSTLTLSKADYEKHKVYACEVTHQGLSSPVTKSFNRGECGGGGSGGGGSGGGGSGGGGSGGGGSGGGGSGGGGSGGGGSQVQLVQSGAEVAKPGASVKMSCKASGYTFTRNTMHWIKQAPGQCLEWIGFIDPHNTYTRYNQKFKDRATLTADTSASTAYMELSSLRSEDTAVYYCARWPMDYWGQGTLVTVSSASTKGPSVFPLAPCSRSTSESTAALGCLVKDYFPEPVTVSWNSGALTSGVHTFPAVLQSSGLYSLSSVVTVPSSSLGTKTYTCNVDHKPSNTKVDKRVESKYGPPCPPCPAPEFLGGPSVFLFPPKPKDTLMISRTPEVTCVVVDVSQEDPEVQFNWYVDGVEVHNAKTKPREEQFNSTYRVVSVLTVLHQDWLNGKEYKCKVSNKGLPSSIEKTISKAKGQPREPQVCTLPPSQEEMTKNQVSLSCAVKGFYPSDIAVEWESNGQPENNYKTTPPVLDSDGSFFLVSRLTVDKSRWQEGNVFSCSVMHEALHNHYTQKSLSLSLGK

SEQ ID NO: 110 - protein, 704 aa, Artificial Sequence
  PL1642-T2353-scFv-HC-PHR protein
QVQLVQSGAEVAKPGASVKMSCKASGYTFTRNTMHWIKQAPGQRLEWIGFIDPHNTYTRYNQKFKDRATLTADTSASTAYMELSSLRSEDTAVYYCARWPMDYWGQGTLVTVSSASTKGPSVFPLAPCSRSTSESTAALGCLVKDYFPEPVTVSWNSGALTSGVHTFPAVLQSSGLYSLSSVVTVPSSSLGTKTYTCNVDHKPSNTKVDKRVESKYGPPCPPCPAPEFEGGPSVFLFPPKPKDTLMISRTPEVTCVVVDVSQEDPEVQFNWYVDGVEVHNAKTKPREEQFNSTYRVVSVLTVLHQDWLNGKEYKCKVSNKGLPSSIEKTISKAKGQPREPQVYTLPPSQEEMTKNQVSLTCLVKGFYPSDIAVEWESNGQPENNYKTTPPVLDSDGSFFLYSRLTVDKSRWQEGNVFSCSVMHEALHNHYTQKSLSLSLGKGGGGSGGGGSEVQLVESGGGLVQPGGSLRLSCAASGFTFSDHWMSWVRQAPGKCMEWIGNIQYDGSYTNYAPSLKNRFTISRDNAKNSLYLQMNSLRAEDTATYYCTRGHFRITMASMGASASVYWGQGTMVTVSSGGGGSGGGGSGGGGSGGGGSDIQMTQSPSSLSASVGDRVTITCRTSQDIGNSLRWFQQKPGKAPKLLIHGATNLANGVPSRFSGSGSGTDFTLTISSLQPEDFATYYCLQHNEYPLTFGCGTKLEIK

SEQ ID NO: 111 - protein, 222 aa, Artificial Sequence
  HuPL1642-VL2-PHR protein
DIVMTQSPDSLAVSLGERVTMRCKSSQSLSWSENQNNYLSWYQQKPGQPPKLLIYGASIRESGVPDRFSGSGSGTDFTLTISSVQAEDVGVYYCQHNHGSFLPYTFGQGTKLEIKRTVAAPSVFIFPPSDEQLKSGTASVVCLLNNFYPREAKVQWKVDNALQSGNSQESVTEQDSKDSTYSLSSTLTLSKADYEKHKVYACEVTHQGLSSPVTKSFNRGEC